European Patent Application EP 4 624 495 A1, published October 1, 2025. Title: ANTIBODIES SPECIFICALLY BINDING TO ASM PROTEIN. Applicant: ISU ABXIS CO., LTD. The sequence listing filed with the application follows.

SEQUENCE LISTING (143 sequences)

SEQ ID NO: 1 - protein, 116 aa, synthetic construct
EVQLLESGGGLVQPGGSLRLSCAASGFTFSNYYMSWVRQAPGKGLEWVSGIYYGSGNIYYADSVKGRFTISRDNSKNTLYLQMNSLRAEDTAVYYCARDTPGFDYWGQGTLVTVSS

SEQ ID NO: 2 - DNA, 348 bp, synthetic construct
  source 1..348: mol_type = other DNA
gaggtgcagctgttggagtctgggggaggcttggtacagcctggggggtccctgagactctcctgtgcagcctccggattcaccttctccaactactacatgtcctgggtccgacaggcccctggcaaaggattggaatgggtgtccggcatctactacggctccggcaacatctactatgccgactccgtgaagggcagattcaccatctctcgggacaactccaagaacaccctgtacctgcagatgaactccctgagagccgaggacaccgccgtgtactactgcgctagagatacccctggcttcgactattggggccagggcacactggtcaccgtgagctca

SEQ ID NO: 3 - protein, 116 aa, synthetic construct
EVQLLESGGGLVQPGGSLRLSCAASGFTFSNYYMSWVRQAPGKGLEWVSGIYFGSGDIRYADSVKGRFTISRDNSKNTLYLQMNSLRAEDTAVYYCARDTPGFDYWGQGTLVTVSS

SEQ ID NO: 4 - DNA, 348 bp, synthetic construct
  source 1..348: mol_type = other DNA
gaggtgcagctgttggagtctgggggaggcttggtacagcctggagggtccctgagactctcctgtgcagcctccggattcacctttagcaattattatatgagctgggtccgccaggctccagggaaggggctggagtgggtctcagggatctattttggtagtggtgatataaggtacgctgattctgtaaaaggtcggttcaccatctccagagacaattccaagaacacgctgtatctgcaaatgaacagcctgagagccgaggacacggccgtgtattactgtgcgagagatacgcctgggttcgactactggggccagggtacactggtcaccgtgagctca

SEQ ID NO: 5 - protein, 116 aa, synthetic construct
EVQLLESGGGLVQPGGSLRLSCAASGFTFSNYYMSWVRQAPGKGLEWVSGIYYGGVKIYYADSVKGRFTISRDNSKNTLYLQMNSLRAEDTAVYYCARDTPGFDYWGQGTLVTVSS

SEQ ID NO: 6 - DNA, 348 bp, synthetic construct
  source 1..348: mol_type = other DNA
gaggtgcagctgttggagtctgggggaggcttggtacagcctggggggtccctgagactctcctgtgcagcctccggattcacctttagcaattattatatgagctgggtccgccaggctccagggaaggggctggagtgggtctcagggatctattatggtggtgttaaaatatattacgctgattctgtaaaaggtcggttcaccatctccagagacaattccaagaacacgctgtatctgcaaatgaacagcctgagagccgaggacacggccgtgtattactgtgcgagagatacgcctgggttcgactactggggccagggtacactggtcaccgtgagctca

SEQ ID NO: 7 - protein, 116 aa, synthetic construct
EVQLLESGGGLVQPGGSLRLSCAASGFTFSNYYMSWVRQAPGKGLEWVSGIYYGNGIPYYADSVKDRFTISRDNSKNTLYLQMNSLRAEDTAVYYCARDTPGFDYWGQGTLVTVSS

SEQ ID NO: 8 - DNA, 348 bp, synthetic construct
  source 1..348: mol_type = other DNA
gaggtgcagctgttggagtctgggggaggcttggtacagcctggggggtccctgagactctcctgtgcagcctccggattcacctttagcaattattatatgagctgggtccgccaggctccagggaaggggctggagtgggtctcaggtatctattatggtaatggtattccatattacgctgattctgtaaaagatcggttcaccatctccagagacaattccaagaacacgctgtatctgcaaatgaacagcctgagagccgaggacacggccgtgtattactgtgcgagagatacgcctgggttcgactactggggccagggtacactggtcaccgtgagctca

SEQ ID NO: 9 - protein, 116 aa, synthetic construct
EVQLLESGGGLVQPGGSLRLSCAASGFTFSNYYMSWVRQAPGKGLEWVSGIYYGSGIPYYADSVKERFTISRDNSKNTLYLQMNSLRAEDTAVYYCARDTPGFDYWGQGTLVTVSS

SEQ ID NO: 10 - DNA, 348 bp, synthetic construct
  source 1..348: mol_type = other DNA
gaggtgcagctgttggagtctgggggaggcttggtacagcctggggggtccctgagactctcctgtgcagcctccggattcacctttagcaattattatatgagctgggtccgccaggctccagggaaggggctggagtgggtctcagggatctattatggtagtggtattccatattacgctgattctgtaaaagaacggttcaccatctccagagacaattccaagaacacgctgtatctgcaaatgaacagcctgagagccgaggacacggccgtgtattactgtgcgagagatacgcctgggttcgactactggggccagggtacactggtcaccgtgagctca

SEQ ID NO: 11 - protein, 116 aa, synthetic construct
EVQLLESGGGLVQPGGSLRLSCAASGFTFSNYYMSWVRQAPGKGLEWVSGIYYGSGIPYYANSVKGRFTISRDNSKNTLYLQMNSLRAEDTAVYYCARDTPGFDYWGQGTLVTVSS

SEQ ID NO: 12 - DNA, 348 bp, synthetic construct
  source 1..348: mol_type = other DNA
gaggtgcagctgttggagtctgggggaggcttggtacagcctggggggtccctgagactctcctgtgcagcctccggattcacctttagcaattattatatgagctgggtccgccaggctccagggaaggggctggagtgggtctcagggatctattatggtagtggtataccctattacgctaattctgtaaaaggtcggttcaccatctccagagacaattccaagaacacgctgtatctgcaaatgaacagcctgagagccgaggacacggccgtgtattactgtgcgagagatacgcctgggttcgactactggggccagggtacactggtcaccgtgagctca

SEQ ID NO: 13 - protein, 116 aa, synthetic construct
EVQLLESGGGLVQPGGSLRLSCAASGFTFSNYYMSWVRQAPGKGLEWVSGIYYGSGKPYYADSVKGRFTISRDNSKNTLYLQMNSLRAEDTAVYYCARDTPGFDYWGQGTLVTVSS

SEQ ID NO: 14 - DNA, 348 bp, synthetic construct
  source 1..348: mol_type = other DNA
gaggtgcagctgttggagtctgggggaggcttggtacagcctggggggtccctgagactctcctgtgcagcctccggattcacctttagcaattattatatgagctgggtccgccaggctccagggaaggggctggagtgggtctcagggatctattatggtagtggtaaaccatattacgctgattctgtaaaaggtcggttcaccatctccagagacaattccaagaacacgctgtatctgcaaatgaacagcctgagagccgaggacacggccgtgtattactgtgcgagagatacgcctgggttcgactactggggccagggtacactggtcaccgtgagctca

SEQ ID NO: 15 - protein, 116 aa, synthetic construct
EVQLLESGGGLVQPGGSLRLSCAASGFTFSNYYMSWVRRAPGKGLEWVSGIYYGSGTPYYAASVKGRFTISRDNSKNTLYLQMNSLRAEDTAVYYCARDTPGFDYWGQGTLVTVSS

SEQ ID NO: 16 - DNA, 348 bp, synthetic construct
  source 1..348: mol_type = other DNA
gaggtgcagctgttggagtctgggggaggcttggtacagcctggggggtccctgagactctcctgtgcagcctccggattcacctttagcaattattatatgagctgggtccgccgggctccagggaaggggctggagtgggtctcagggatctattatggtagtggtactccatattacgctgcttctgtaaaaggtcggttcaccatctccagagacaattccaagaacacgctgtatctgcaaatgaacagcctgagagccgaggacacggccgtgtattactgtgcgagagatacgcctgggttcgactactggggccagggtacactggtcaccgtgagctca

SEQ ID NO: 17 - protein, 116 aa, synthetic construct
EVQLLESGGGLVQPGGSLRLSCAASGFTFSNYYMSWVRQAPGKGLEWVSGIYYGSGTPYYSDSVKGRFTISRDNSKNTLYLQMNSLRAEDTAVYYCARDTPGFDYWGQGTLVTVSS

SEQ ID NO: 18 - DNA, 348 bp, synthetic construct
  source 1..348: mol_type = other DNA
gaggtgcagctgttggagtctgggggaggcttggtacagcctggggggtccctgagactctcctgtgcagcctccggattcacctttagcaattattatatgagctgggtccgccaggctccagggaaggggctggagtgggtctcagggatctactatggtagtggtactccatactactctgactctgtaaaaggtcggttcaccatctccagagacaattccaagaacacgctgtatctgcaaatgaacagcctgagagccgaggacacggccgtgtattactgtgcgagagatacgcctgggttcgactactggggccagggtacactggtcaccgtgagctca

SEQ ID NO: 19 - protein, 116 aa, synthetic construct
EVQLLESGGGLVQPGGSLRLSCAASGFTFSNYYMSWVRQAPGKGLEWVSGIYYGSGVPYYADSVKGRFTISRDNSKNTLYLQMNSLRAEDTAVYYCARDTPGFDYWGQGTLVTVSS

SEQ ID NO: 20 - DNA, 348 bp, synthetic construct
  source 1..348: mol_type = other DNA
gaggtgcagctgttggagtctgggggaggcttggtacagcctggggggtccctgagactctcctgtgcagcctccggattcacctttagcaattattatatgagctgggtccgccaggctccagggaaggggctggagtgggtctcagggatctactatggcagtggtgttccatattacgctgattctgtcaaagggcggttcaccatctccagagacaattccaagaacacgctgtatctgcaaatgaacagcctgagagccgaggacacggccgtgtattactgtgcgagagatacgcctgggttcgactactggggccagggtacactggtcaccgtgagctca

SEQ ID NO: 21 - protein, 116 aa, synthetic construct
EVQLLESGGGLVQPGGSLRLSCAASGFTFSNYYMSWVRQAPGKGLEWVSGLYYGGGTPYYADSVKGRFTISRDNSKNTLYLQMNSLRAEDTAVYYCARDTPGFDYWGQGTLVTVSS

SEQ ID NO: 22 - DNA, 348 bp, synthetic construct
  source 1..348: mol_type = other DNA
gaggtgcagctgttggagtctgggggaggcttggtacagcctggggggtccctgagactctcctgtgcagcctccggattcacctttagcaattattatatgagctgggtccgccaggctccagggaaggggctggagtgggtctcagggctctattatggtggtggtactccatattacgctgattctgtaaaaggtcggttcaccatctccagagacaattccaagaacacgctgtatctgcaaatgaacagcctgagagctgaggacacggccgtgtattactgtgcgagagatacgcctgggttcgactactggggccagggtacactggtcaccgtgagctca

SEQ ID NO: 23 - protein, 116 aa, synthetic construct
EVQLLESGGGLVQPGGSLRLSCAASGFTFSNYYMSWVRQAPGKGLEWVSGLYYGSGIPYYADSVKGRFTISRDNSKNTLYLQMNSLRAEDTAVYYCARDTPGFDYWGQGTLVTVSS

SEQ ID NO: 24 - DNA, 348 bp, synthetic construct
  source 1..348: mol_type = other DNA
gaggtgcagctgttggagtctgggggaggcttggtacagcctggggggtccctgagactctcctgtgcagcctccggattcacctttagcaattattatatgagctgggtccgccaggctccagggaaggggctggagtgggtctcagggttgtattatggtagtggtattccatattacgctgattctgtaaaaggtcggttcaccatctccagagacaattccaagaacacgctgtatctgcaaatgaacagcctgagagccgaggacacggccgtgtattactgtgcgagagatacgcctgggttcgactactggggccagggtacactggtcaccgtgagctca

SEQ ID NO: 25 - protein, 116 aa, synthetic construct
EVQLLESGGGLVQPGGSLRLSCAASGFTFSNYYMSWVRQAPGKGLEWVSGTYYASGGIYYADSVKGRFTISRDNSKNTLYLQMNSLRAEDTAVYYCARDTPGFDYWGQGTLVTVSS

SEQ ID NO: 26 - DNA, 348 bp, synthetic construct
  source 1..348: mol_type = other DNA
gaggtgcagctgttggagtctgggggaggcttggtacagcctggggggtccctgagactctcctgtgcagcctccggattcacctttagcaattattatatgagctgggtccgccaggctccagggaaggggctggagtgggtctcagggacatattatgctagtggtggtatatattacgctgattctgtaaaaggtcggttcaccatctccagagacaattccaagaacacgctgtatctgcaaatgaacagcctgagagccgaggacacggccgtgtattactgtgcgagagatacgcctgggttcgactactggggccagggtacactggtcaccgtgagctca

SEQ ID NO: 27 - protein, 116 aa, synthetic construct
EVQLLESGGGLVQPGGSLRLSCAASGFTFSNYYMSWVRQAPGKGLEWVSGTYYASGNAYYADSVKGRFTISRDNSKNTLYLQMNSLRAEDTAVYYCARDTPGFDYWGQGTLVTVSS

SEQ ID NO: 28 - DNA, 348 bp, synthetic construct
  source 1..348: mol_type = other DNA
gaggtgcagctgttggagtctgggggaggcttggtacagcctggggggtccctgagactctcctgtgcagcctccggattcacctttagcaattattatatgagctgggtccgccaggctccagggaaggggctggagtgggtctcagggacctattatgctagtggtaatgcatattacgctgattctgtaaaaggtcggttcaccatctccagagacaattccaagaacacgctgtatctgcaaatgaacagcctgagagccgaggacacggccgtgtattactgtgcgagagatacgcctgggttcgactactggggccagggtacactggtcaccgtgagctca

SEQ ID NO: 29 - protein, 116 aa, synthetic construct
EVQLLESGGGLVQPGGSLRLSCAASGFTFSNYYMSWVRQAPGKGLEWVSGTYYDSGYVYYADSVKGRFTISRDNSKNTLYLQMNSLRAEDTAVYYCARDTPGFDYWGQGTLVTVSS

SEQ ID NO: 30 - DNA, 348 bp, synthetic construct
  source 1..348: mol_type = other DNA
gaggtgcagctgttggagtctgggggaggcttggtacagcctggggggtccctgagactctcctgtgcagcctccgggttcacctttagcaattattatatgagctgggtccgccaggctccagggaaggggctggagtgggtctcagggacctattatgatagtggatatgtatattacgctgattctgtaaaaggtcggttcaccatctccagagacaattccaagaacacgctgtatctgcaaatgaacagcctgagagccgaggacacggccgtgtattactgtgcgagagatacgcctgggttcgactactggggccagggtacactggtcaccgtgagctca

SEQ ID NO: 31 - protein, 116 aa, synthetic construct
EVQLLESGGGLVQPGGSLRLSCAASGFTFSNYYMSWVRQAPGKGLEWVSGTYYSSGGIYYADSVKGRFTISRDNSKNTLYLQMNSLRAEDTAVYYCARDTPGFDYWGQGTLVTVSS

SEQ ID NO: 32 - DNA, 348 bp, synthetic construct
  source 1..348: mol_type = other DNA
gaggtgcagctgttggagtctgggggaggcttggtacagcctggggggtccctgagactctcctgtgcagcctccggattcacctttagcaattattatatgagctgggtccgccaggctccagggaaggggctggagtgggtctcagggacctattatagtagtggtggtatatattacgctgattctgtcaaaggccggttcaccatctccagagacaattccaagaacacgctgtatctgcaaatgaacagcctgagagccgaggacacggccgtgtattactgtgcgagagatacgcctgggttcgactactggggccagggtacactggtcaccgtgagctca

SEQ ID NO: 33 - protein, 116 aa, synthetic construct
EVQLLESGGGLVQPGGSLRLSCAASGFTFSNYYMSWVRQAPGKGLEWVSGVYYGSGTPYYADSVKGRFTISRDNSKNTLYLQMNSLRAEDTAVYYCARDTPGFDYWGQGTLVTVSS

SEQ ID NO: 34 - DNA, 348 bp, synthetic construct
  source 1..348: mol_type = other DNA
gaggtgcagctgttggagtctgggggaggcttggtacagcctggggggtccctgagactctcctgtgcagcctccggattcacctttagcaattattatatgagctgggtccgccaggctccagggaaggggctggagtgggtctcaggggtctactatggtagtggtactccatattacgctgattctgtaaaaggtcggttcaccatctccagagacaattccaagaacacgctgtatctgcaaatgaacagcctgagagccgaggacacggccgtgtattactgtgcgagagatacgcctgggttcgactactggggccagggtacactggtcaccgtgagctca

SEQ ID NO: 35 - protein, 116 aa, synthetic construct
EVQLLESGGGLVQPGGSLRLSCAASGFTFSNYYMSWVRQAPGKGLEWVSGVYYPSGNPYYADSVKGRFTISRDNSKNTLYLQMNSLRAEDTAVYYCARDTPGFDYWGQGTLVTVSS

SEQ ID NO: 36 - DNA, 348 bp, synthetic construct
  source 1..348: mol_type = other DNA
gaggtgcagctgttggagtctgggggaggcttggtacagcctggggggtccctgagactctcctgtgcagcctccggattcacctttagcaattattatatgagctgggtccgccaggctccagggaaggggctggagtgggtctcaggggtatattatcctagtggtaatccatattacgctgattctgttaaaggtcggttcaccatctccagagacaattccaagaacacgctgtatctgcaaatgaacagcctgagagccgaggacacggccgtgtattactgtgcgagagatacgcctgggttcgactactggggccagggtacactggtcaccgtgagctca

SEQ ID NO: 37 - protein, 110 aa, synthetic construct
QSVLTQPPSASGTPGQRVTISCTGSSSNIGNNAVNWYQQLPGTAPKLLIYYDSHRPSGVPDRFSGSKSGTSASLAISGLRSEDEADYYCGAWDYSLSAYVFGGGTKLTVL

SEQ ID NO: 38 - DNA, 330 bp, synthetic construct
  source 1..330: mol_type = other DNA
cagtctgtgctgactcagccaccctcagctagcggcacacctggccagagagtgaccatctcttgtaccggctcctcctccaacatcggcaacaacgccgtgaactggtatcagcagctgcctggcacagcccctaaactgctgatctactacgactcccaccggcctagcggcgtgcccgatagattttccggctctaagtccggcacctctgccagcctggctatctctggactgagatctgaggacgaggccgactactactgtggcgcctgggactactctctgtccgcctatgtttttggcggaggcaccaagcttacggtccta

SEQ ID NO: 39 - protein, 110 aa, synthetic construct
QSVLTQPPSASGTPGQRVTISCTGSSSNIGNNAVNWYQQLPGTAPKLLIYYDIFQPSGVPDRFSGSKSGTSASLAISGLRSEDEADYYCGAWDYSLSAYVFGGGTKLTVL

SEQ ID NO: 40 - DNA, 330 bp, synthetic construct
  source 1..330: mol_type = other DNA
cagtctgtgctgactcagccaccctcagctagcgggacccccgggcagagggtcaccatctcttgtactggctcttcatctaatattggcaataatgctgtcaactggtaccagcagctcccaggaacggcccccaaactcctcatctattatgatatttttcagccaagcggggtccctgaccgattctctggctccaagtctggcacctcagcctccctggccatcagtgggctccggtccgaggatgaggctgattattactgtggtgcttgggattatagcctgagtgcttatgtcttcggcggaggcaccaagcttacggtccta

SEQ ID NO: 41 - protein, 110 aa, synthetic construct
QSVLTQPPSASGTPGQRVTISCTGSSSNIGNNAVNWYQQLPGTAPKLLIYYDIFRPDGVPDRFSGSKSGTSASLAISGLRSEDEADYYCGAWDYSLSAYVFGGGTKLTVL

SEQ ID NO: 42 - DNA, 330 bp, synthetic construct
  source 1..330: mol_type = other DNA
cagtctgtgctgactcagccaccctcagctagcgggacccccgggcagagggtcaccatctcttgtactggctcttcatctaatattggcaataatgctgtcaactggtaccagcagctcccaggaacggcccccaaactcctcatctattatgatatttttcggccagacggggtccctgaccgattctctggctccaagtctggcacctcagcctccctggccatcagtgggctccggtccgaggatgaggctgattattactgtggtgcttgggattatagcctgagtgcttatgtcttcggcggaggcaccaagcttacggtccta

SEQ ID NO: 43 - protein, 110 aa, synthetic construct
QSVLTQPPSASGTPGQRVTISCTGSSSNIGNNAVNWYQQLPGTAPKLLIYYDIHRPYGVPDRFSGSKSGTSASLAISGLRSEDEADYYCGAWDYSLSAYVFGGGTKLTVL

SEQ ID NO: 44 - DNA, 330 bp, synthetic construct
  source 1..330: mol_type = other DNA
cagtctgtgctgactcagccaccctcagctagcgggacccccgggcagagggtcaccatctcttgtactggctcttcatctaatattggcaataatgctgtcaactggtaccagcagctcccaggaacggcccccaaactcctcatctattatgatattcatcggccatacggggtccctgaccgattctctggctccaagtctggcacctcagcctccctggccatcagtgggctccggtccgaggatgaggctgattattactgtggtgcttgggattatagcctgagtgcttatgtcttcggcggaggcaccaagcttacggtccta

SEQ ID NO: 45 - protein, 110 aa, synthetic construct
QSVLTQPPSASGTPGQRVTISCTGSSSNIGNNAVNWYQQLPGTAPKLLIYYDLFRPSGVPDRFSGSKSGTSASLAISGLRSEDEADYYCGAWDYSLSAYVFGGGTKLTVL

SEQ ID NO: 46 - DNA, 330 bp, synthetic construct
  source 1..330: mol_type = other DNA
cagtctgtgctgactcagccaccctcagctagcgggacccccgggcagagggtcaccatctcttgtactggctcttcatctaatattggcaataatgctgtcaactggtaccagcagctcccaggaacggcccccaaactcctcatctattatgatctttttaggccaagcggggtccctgaccgattctctggctccaagtctggcacctcagcctccctggccatcagtgggctccggtccgaggatgaggctgattattactgtggtgcttgggattatagcctgagtgcttatgtcttcggcggaggcaccaagcttacggtccta

SEQ ID NO: 47 - protein, 110 aa, synthetic construct
QSVLTQPPSASGTPGQRVTISCTGSSSNIGNNAVNWYQQLPGTAPKLLIYYDMFRPGGVPDRFSGSKSGTSASLAISGLRSEDEADYYCGAWDYSLSAYVFGGGTKLTVL

SEQ ID NO: 48 - DNA, 330 bp, synthetic construct
  source 1..330: mol_type = other DNA
cagtctgtgctgactcagccaccctcagctagcgggacccccgggcagagggtcaccatctcttgtactggctcttcatctaatattggcaataatgctgtcaactggtaccagcagctcccaggaacggcccccaaactcctcatctattacgatatgttccggccaggcggggtccctgaccgattctctggctccaagtctggcacctcagcctccctggccatcagtgggctccggtccgaggatgaggctgattattactgtggtgcttgggattatagcctgagtgcttatgtcttcggcggaggcaccaagcttacggtccta

SEQ ID NO: 49 - protein, 110 aa, synthetic construct
QSVLTQPPSASGTPGQRVTISCTGSSSNIGNNAVNWYQQLPGTAPKLLIYYDMFRPNGVPDRFSGSKSGTSASLAISGLRSEDEADYYCGAWDYSLSAYVFGGGTKLTVL

SEQ ID NO: 50 - DNA, 330 bp, synthetic construct
  source 1..330: mol_type = other DNA
cagtctgtgctgactcagccaccctcagctagcgggacccccgggcagagggtcaccatctcttgtactggctcttcatctaatattggcaataatgctgtcaactggtaccagcagctcccaggaacggcccccaaactcctcatctattatgatatgttccggccaaacggggtccctgaccgattctctggctccaagtctggcacctcagcctccctggccatcagtgggctccggtccgaggatgaggctgattattactgtggtgcttgggattatagcctgagtgcttatgtcttcggcggaggcaccaagcttacggtccta

SEQ ID NO: 51 - protein, 110 aa, synthetic construct
QSVLTQPPSASGTPGQRVTISCTGSSSNIGNNAVNWYQQLPGTAPKLLIYYDQFRPSGVPDRFSGSKSGTSASLAISGLRSEDEADYYCGAWDYSLSAYVFGGGTKLTVL

SEQ ID NO: 52 - DNA, 330 bp, synthetic construct
  source 1..330: mol_type = other DNA
cagtctgtgctgactcagccaccctcagctagcgggacccccgggcagagggtcaccatctcttgtactggctcttcatctaatattggcaataatgctgtcaactggtaccagcagctcccaggaacggcccccaaactcctcatctattatgatcaatttcggccaagcggggtccctgaccgattctctggctccaagtctggcacctcagcctccctggccatcagtgggctccggtccgaggatgaggctgattattactgtggtgcttgggattatagcctgagtgcttatgtcttcggcggaggcaccaagcttacggtccta

SEQ ID NO: 53 - protein, 110 aa, synthetic construct
QSVLTQPPSASGTPGQRVTISCTGSSSNIGNNAVNWYQQLPGTAPKLLIYYDSFPASGVPDRFSGSKSGTSASLAISGLRSEDEADYYCGAWDYSLSAYVFGGGTKLTVL

SEQ ID NO: 54 - DNA, 330 bp, synthetic construct
  source 1..330: mol_type = other DNA
cagtctgtgctgactcagccaccctcagctagcgggacccccgggcagagggtcaccatctcttgtactggctcttcatctaatattggcaataatgctgtcaactggtaccagcagctcccaggaacggcccccaaactcctcatctattatgatagttttccggcaagcggggtccctgaccgattctctggctccaagtctggcacctcagcctccctggccatcagtgggctccggtccgaggatgaggctgattattactgtggtgcttgggattatagcctgagtgcttatgtcttcggcggaggcaccaagcttacggtccta

SEQ ID NO: 55 - protein, 110 aa, synthetic construct
QSVLTQPPSASGTPGQRVTISCTGSSSNIGNNAVNWYQQLPGTAPKLLIYYDSFRQSGVPDRFSGSKSGTSASLAISGLRSEDEADYYCGAWDYSLSAYVFGGGTKLTVL

SEQ ID NO: 56 - DNA, 330 bp, synthetic construct
  source 1..330: mol_type = other DNA
cagtctgtgctgactcagccaccctcagctagcgggacccccgggcagagggtcaccatctcttgtactggctcttcatctaatattggcaataatgctgtcaactggtaccagcagctcccaggaacggcccccaaactcctcatctattatgatagttttcggcaaagcggggtccctgaccgattctctggctccaagtctggcacctcagcctccctggccatcagtgggctccggtccgaggatgaggctgattattactgtggtgcttgggattatagcctgagtgcttatgtcttcggcggaggcaccaagcttacggtccta

SEQ ID NO: 57 - protein, 110 aa, synthetic construct
QSVLTQPPSASGTPGQRVTISCTGSSSNIGNNAVNWYQQLPGTAPKLLIYYDSFRRSGVPDRFSGSKSGTSASLAISGLRSEDEADYYCGAWDYSLSAYVFGGGTKLTVL

SEQ ID NO: 58 - DNA, 330 bp, synthetic construct
  source 1..330: mol_type = other DNA
cagtctgtgctgactcagccaccctcagctagcgggacccccgggcagagggtcaccatctcttgtactggctcttcatctaatattggcaataatgctgtcaactggtaccagcagctcccaggaacggcccccaaactcctcatctattatgatagttttcggcgaagcggggtccctgaccgattctctggctccaagtctggcacctcagcctccctggccatcagtgggctccggtccgaggatgaggctgattattactgtggtgcttgggattatagcctgagtgcttatgtcttcggcggaggcaccaagcttacggtccta

SEQ ID NO: 59 - protein, 110 aa, synthetic construct
QSVLTQPPSASGTPGQRVTISCTGSSSNIGNNAVNWYQQLPGTAPKLLIYYDSFRSTGVPDRFSGSKSGTSASLAISGLRSEDEADYYCGAWDYSLSAYVFGGGTKLTVL

SEQ ID NO: 60 - DNA, 330 bp, synthetic construct
  source 1..330: mol_type = other DNA
cagtctgtgctgactcagccaccctcagctagcgggacccccgggcagagggtcaccatctcttgtactggctcttcatctaatattggcaataatgctgtcaactggtaccagcagctcccaggaacggcccccaaactcctcatctattacgatagttttcggtcaaccggggtccctgaccgattctctggctccaagtctggcacctcagcctccctggccatcagtgggctccggtccgaggatgaggctgattattactgtggtgcttgggattatagcctgagtgcttatgtcttcggcggaggcaccaagcttacggtccta

SEQ ID NO: 61 - protein, 110 aa, synthetic construct
QSVLTQPPSASGTPGQRVTISCTGSSSNIGNNAVNWYQQLPGTAPKLLIYYDSYLPSGVPDRFSGSKSGTSASLAISGLRSEDEADYYCGAWDYSLSAYVFGGGTKLTVL

SEQ ID NO: 62 - DNA, 330 bp, synthetic construct
  source 1..330: mol_type = other DNA
cagtctgtgctgactcagccaccctcagctagcgggacccccgggcagagggtcaccatctcttgtactggctcttcatctaatattggcaataatgctgtcaactggtaccagcagctcccaggaacggcccccaaactcctcatctattatgatagttatctgccaagcggggtccctgaccgattctctggctccaagtctggcacctcagcctccctggccatcagtgggctccggtccgaggatgaggctgattattactgtggtgcttgggattatagcctgagtgcttatgtcttcggcggaggcaccaagcttacggtccta

SEQ ID NO: 63 - protein, 110 aa, synthetic construct
QSVLTQPPSASGTPGQRVTISCTGSSSNIGNNAVNWYQQLPGTAPKLLIYYDSYPPYGVPDRFSGSKSGTSASLAISGLRSEDEADYYCGAWDYSLSAYVFGGGTKLTVL

SEQ ID NO: 64 - DNA, 330 bp, synthetic construct
  source 1..330: mol_type = other DNA
cagtctgtgctgactcagccaccctcagctagcgggacccccgggcagagggtcaccatctcttgtactggctcttcatctaatattggcaataatgctgtcaactggtaccagcagctcccaggaacggcccccaaactcctcatctattatgatagttatccgccatacggggtccctgaccgattctctggctccaagtctggcacctcagcctccctggccatcagtgggctccggtccgaggatgaggctgattattactgtggtgcttgggattatagcctgagtgcttatgtcttcggcggaggcaccaagcttacggtccta

SEQ ID NO: 65 - protein, 110 aa, synthetic construct
QSVLTQPPSASGTPGQRVTISCTGSSSNIGNNAVNWYQQLPGTAPKLLIYYDSYQASGVPDRFSGSKSGTSASLAISGLRSEDEADYYCGAWDYSLSAYVFGGGTKLTVL

SEQ ID NO: 66 - DNA, 330 bp, synthetic construct
  source 1..330: mol_type = other DNA
cagtctgtgctgactcagccaccctcagctagcgggacccccgggcagagggtcaccatctcttgtactggctcttcatctaatattggcaataatgctgtcaactggtaccagcagctcccaggaacggcccccaaactcctcatctattatgatagttatcaggcaagcggggtccctgaccgattctctggctccaagtctggcacctcagcctccctggccatcagtgggctccggtccgaggatgaggctgattattactgtggtgcttgggattatagcctgagtgcttatgtcttcggcggaggcaccaagcttacggtccta

SEQ ID NO: 67 - protein, 110 aa, synthetic construct
QSVLTQPPSASGTPGQRVTISCTGSSSNIGNNAVNWYQQLPGTAPKLLIYYDSYRASGVPDRFSGSKSGTSASLAISGLRSEDEADYYCGAWDYSLSAYVFGGGTKLTVL

SEQ ID NO: 68 - DNA, 330 bp, synthetic construct
  source 1..330: mol_type = other DNA
cagtctgtgctgactcagccaccctcagctagcgggacccccgggcagagggtcaccatctcttgtactggctcttcatctaatattggcaataatgctgtcaactggtaccagcagctcccaggaacggcccccaaactcctcatctattatgatagttatcgggcaagcggggtccctgaccgattctctggctccaagtctggcacctcagcctccctggccatcagtgggctccggtccgaggatgaggctgattattactgtggtgcttgggattatagcctgagtgcttatgtcttcggcggaggcaccaagcttacggtccta

SEQ ID NO: 69 - protein, 110 aa, synthetic construct
QSVLTQPPSASGTPGQRVTISCTGSSSNIGNNAVNWYQQLPGTAPKLLIYYDSYRPFGVPDRFSGSKSGTSASLAISGLRSEDEADYYCGAWDYSLSAYVFGGGTKLTVL

SEQ ID NO: 70 - DNA, 330 bp, synthetic construct
  source 1..330: mol_type = other DNA
cagtctgtgctgactcagccaccctcagctagcgggacccccgggcagagggtcaccatctcttgtactggctcttcatctaatattggcaataatgctgtcaactggtaccagcagctcccaggaacggcccccaaactcctcatctattatgatagttatcggccattcggggtccctgaccgattctctggctccaagtctggcacctcagcctccctggccatcagtgggctccggtccgaggatgaggctgattattactgtggtgcttgggattatagcctgagtgcttatgtcttcggcggaggcaccaagcttacggtccta

SEQ ID NO: 71 - protein, 110 aa, synthetic construct
QSVLTQPPSASGTPGQRVTISCTGSSSNIGNNAVNWYQQLPGTAPKLLIYYDSYRPGGVPDRFSGSKSGTSASLAISGLRSEDEADYYCGAWDYSLSAYVFGGGTKLTVL

SEQ ID NO: 72 - DNA, 330 bp, synthetic construct
  source 1..330: mol_type = other DNA
cagtctgtgctgactcagccaccctcagctagcgggacccccgggcagagggtcaccatctcttgtactggctcttcatctaatattggcaataatgctgtcaactggtaccagcagctcccaggaacggcccccaaactcctcatctattatgacagttatcggccagggggggtccctgaccgattctctggctccaagtctggcacctcagcctccctggccatcagtgggctccggtccgaggatgaggctgattattactgtggtgcttgggattatagcctgagtgcttatgtcttcggcggaggcaccaagcttacggtccta

SEQ ID NO: 73 - protein, 110 aa, synthetic construct
QSVLTQPPSASGTPGQRVTISCTGSSSNIGNNAVNWYQQLPGTAPKLLIYYDSYRSWGVPDRFSGSKSGTSASLAISGLRSEDEADYYCGAWDYSLSAYVFGGGTKLTVL

SEQ ID NO: 74 - DNA, 330 bp, synthetic construct
  source 1..330: mol_type = other DNA
cagtctgtgctgactcagccaccctcagctagcgggacccccgggcagagggtcaccatctcttgtactggctcttcatctaatattggcaataatgctgtcaactggtaccagcagctcccaggaacggcccccaaactcctcatctattatgatagttatcggtcatggggggtccctgaccgattctctggctccaagtctggcacctcagcctccctggccatcagtgggctccggtccgaggatgaggctgattattactgtggtgcttgggattatagcctgagtgcttatgtcttcggcggaggcaccaagcttacggtccta

SEQ ID NO: 75 - protein, 110 aa, synthetic construct
QSVLTQPPSASGTPGQRVTISCTGSSSNIGNNAVNWYQQLPGTAPKLLIYYDSYTPSGVPDRFSGSKSGTSASLAISGLRSEDEADYYCGAWDYSLSAYVFGGGTKLTVL

SEQ ID NO: 76 - DNA, 330 bp, synthetic construct
  source 1..330: mol_type = other DNA
cagtctgtgctgactcagccaccctcagctagcgggacccccgggcagagggtcaccatctcttgtactggctcttcatctaatattggcaataatgctgtcaactggtaccagcagctcccaggaacggcccccaaactcctcatctattatgatagttatacgccaagcggggtccctgaccgattctctggctccaagtctggcacctcagcctccctggccatcagtgggctccggtccgaggatgaggctgattattactgtggtgcttgggattatagcctgagtgcttatgtcttcggcggaggcaccaagcttacggtccta

SEQ ID NO: 77 - protein, 110 aa, synthetic construct
QSVLTQPPSASGTPGQRVTISCTGSSSNIGNNAVNWYQQLPGTAPKLLIYYDTFRPTGVPDRFSGSKSGTSASLAISGLRSEDEADYYCGAWDYSLSAYVFGGGTKLTVL

SEQ ID NO: 78 - DNA, 330 bp, synthetic construct
  source 1..330: mol_type = other DNA
cagtctgtgctgactcagccaccctcagctagcgggacccccgggcagagggtcaccatctcttgtactggctcttcatctaatattggcaataatgctgtcaactggtaccagcagctcccaggaacggcccccaaactcctcatctattatgatactttccggccaaccggggtccctgaccgattctctggctccaagtctggcacctcagcctccctggccatcagtgggctccggtccgaggatgaggctgattattactgtggtgcttgggattatagcctgagtgcttatgtcttcggcggaggcaccaagcttacggtccta

SEQ ID NO: 79 - protein, 110 aa, synthetic construct
QSVLTQPPSASGTPGQRVTISCTGSSSNIGNNAVNWYQQLPGTAPKLLIYYDVHRPRGVPDRFSGSKSGTSASLAISGLRSEDEADYYCGAWDYSLSAYVFGGGTKLTVL

SEQ ID NO: 80 - DNA, 330 bp, synthetic construct
  source 1..330: mol_type = other DNA
cagtctgtgctgactcagccaccctcagctagcgggacccccgggcagagggtcaccatctcttgtactggctcttcatctaatattggcaataatgctgtcaactggtaccagcagctcccaggaacggcccccaaactcctcatctattatgatgttcatcggcccaggggggtccctgaccgattctctggctccaagtctggcacctcagcctccctggccatcagtgggctccggtccgaggatgaggctgattattactgtggtgcttgggattatagcctgagtgcttatgtcttcggcggaggcaccaagcttacggtccta

SEQ ID NO: 81 - protein, 110 aa, synthetic construct
QSVLTQPPSASGTPGQRVTISCTGSSSNIGNNAVNWYQQLPGTAPKLLIYYDWYRPTGVPDRFSGSKSGTSASLAISGLRSEDEADYYCGAWDYSLSAYVFGGGTKLTVL

SEQ ID NO: 82 - DNA, 330 bp, synthetic construct
  source 1..330: mol_type = other DNA
cagtctgtgctgactcagccaccctcagctagcgggacccccgggcagagggtcaccatctcttgtactggctcttcatctaatattggcaataatgctgtcaactggtaccagcagctcccaggaacggcccccaaactcctcatctattatgattggtatcggccaaccggggtccctgaccgattctctggctccaagtctggcacctcagcctccctggccatcagtgggctccggtccgaggatgaggctgattattactgtggtgcttgggattatagcctgagtgcttatgtcttcggcggaggcaccaagcttacggtccta

SEQ ID NO: 83 - protein, 110 aa, synthetic construct
QSVLTQPPSASGTPGQRVTISCTGSSSNIGNNAVNWYQQLPGTAPKLLIYYDSHRPSGVPDRFSGSKSGTSASLAISGLRSEDEADYYCGAWDYWLGAYVFGGGTKLTVL

SEQ ID NO: 84 - DNA, 330 bp, synthetic construct
  source 1..330: mol_type = other DNA
cagtctgtgctgactcagccaccctcagctagcgggacccccgggcagagggtcaccatctcttgtactggctcttcatctaatattggcaataatgctgtcaactggtaccagcagctcccaggaacggcccccaaactcctcatctattatgatagtcatcggccaagcggggtccctgaccgattctctggctccaagtctggcacctcagcctccctggccattagtgggctccggtccgaggatgaggctgattattactgtggtgcttgggattattggctgggtgcttatgtcttcggcggaggcaccaagcttacggtccta

SEQ ID NO: 85 - protein, 110 aa, synthetic construct
QSVLTQPPSASGTPGQRVTISCTGSSSNIGNNAVNWYQQLPGTAPKLLIYYDYFSHSGVPDRFSGSKSGTSASLAISGLRSEDEADYYCGAWDYSLSAYVFGGGTKLTVL

SEQ ID NO: 86 - DNA, 330 bp, synthetic construct
  source 1..330: mol_type = other DNA
cagtctgtgctgactcagccaccctcagctagcgggacccccgggcagagggtcaccatctcttgtactggctcttcatctaatattggcaataatgctgtcaactggtaccagcagctcccaggaacggcccccaaactcctcatctattatgattattttagccatagcggggtccctgaccgattctctggctccaagtctggcacctcagcctccctggccatcagtgggctccggtccgaggatgaggctgattattactgtggtgcttgggattatagcctgagtgcttatgtcttcggcggaggcaccaagcttacggtccta

SEQ ID NO: 87 - protein, 110 aa, synthetic construct
QSVLTQPPSASGTPGQRVTISCTGSSSNIGNNAVNWYQQLPGTAPKLLIYYDYYQSSGVPDRFSGSKSGTSASLAISGLRSEDEADYYCGAWDYSLSAYVFGGGTKLTVL

SEQ ID NO: 88 - DNA, 330 bp, synthetic construct
  source 1..330: mol_type = other DNA
cagtctgtgctgactcagccaccctcagctagcgggacccccgggcagagggtcaccatctcttgtactggctcttcatctaatattggcaataatgctgtcaactggtaccagcagctcccaggaacggcccccaaactcctcatctattatgattattatcagtcaagcggggtccctgaccgattctctggctccaagtctggcacctcagcctccctggccatcagtgggctccggtccgaggatgaggctgattattactgtggtgcttgggattatagcctgagtgcttatgtcttcggcggaggcaccaagcttacggtccta

SEQ ID NO: 89 - protein, 5 aa, synthetic construct
NYYMS

SEQ ID NO: 90 - protein, 17 aa, synthetic construct
GIYYGSGNIYYADSVKG

SEQ ID NO: 91 - protein, 7 aa, synthetic construct
DTPGFDY

SEQ ID NO: 92 - protein, 13 aa, synthetic construct
TGSSSNIGNNAVN

SEQ ID NO: 93 - protein, 7 aa, synthetic construct
YDSHRPS

SEQ ID NO: 94 - protein, 11 aa, synthetic construct
GAWDYSLSAYV

SEQ ID NO: 95 - protein, 17 aa, synthetic construct
GIYFGSGDIRYADSVKG

SEQ ID NO: 96 - protein, 17 aa, synthetic construct
GIYYGGVKIYYADSVKG

SEQ ID NO: 97 - protein, 17 aa, synthetic construct
GIYYGNGIPYYADSVKD

SEQ ID NO: 98 - protein, 17 aa, synthetic construct
GIYYGSGIPYYADSVKE

SEQ ID NO: 99 - protein, 17 aa, synthetic construct
GIYYGSGIPYYANSVKG

SEQ ID NO: 100 - protein, 17 aa, synthetic construct
GIYYGSGKPYYADSVKG

SEQ ID NO: 101 - protein, 17 aa, synthetic construct
GIYYGSGTPYYAASVKG

SEQ ID NO: 102 - protein, 17 aa, synthetic construct
GIYYGSGTPYYSDSVKG

SEQ ID NO: 103 - protein, 17 aa, synthetic construct
GIYYGSGVPYYADSVKG

SEQ ID NO: 104 - protein, 17 aa, synthetic construct
GLYYGGGTPYYADSVKG

SEQ ID NO: 105 - protein, 17 aa, synthetic construct
GLYYGSGIPYYADSVKG

SEQ ID NO: 106 - protein, 17 aa, synthetic construct
GTYYASGGIYYADSVKG

SEQ ID NO: 107 - protein, 17 aa, synthetic construct
GTYYASGNAYYADSVKG

SEQ ID NO: 108 - protein, 17 aa, synthetic construct
GTYYDSGYVYYADSVKG

SEQ ID NO: 109 - protein, 17 aa, synthetic construct
GTYYSSGGIYYADSVKG

SEQ ID NO: 110 - protein, 17 aa, synthetic construct
GVYYGSGTPYYADSVKG

SEQ ID NO: 111 - protein, 17 aa, synthetic construct
GVYYPSGNPYYADSVKG

SEQ ID NO: 112 - protein, 7 aa, synthetic construct
YDIFQPS

SEQ ID NO: 113 - protein, 7 aa, synthetic construct
YDIFRPD

SEQ ID NO: 114 - protein, 7 aa, synthetic construct
YDIHRPY

SEQ ID NO: 115 - protein, 7 aa, synthetic construct
YDLFRPS

SEQ ID NO: 116 - protein, 7 aa, synthetic construct
YDMFRPG

SEQ ID NO: 117 - protein, 7 aa, synthetic construct
YDMFRPN

SEQ ID NO: 118 - protein, 7 aa, synthetic construct
YDQFRPS

SEQ ID NO: 119 - protein, 7 aa, synthetic construct
YDSFPAS

SEQ ID NO: 120 - protein, 7 aa, synthetic construct
YDSFRQS

SEQ ID NO: 121 - protein, 7 aa, synthetic construct
YDSFRRS

SEQ ID NO: 122 - protein, 7 aa, synthetic construct
YDSFRST

SEQ ID NO: 123 - protein, 7 aa, synthetic construct
YDSYLPS

SEQ ID NO: 124 - protein, 7 aa, synthetic construct
YDSYPPY

SEQ ID NO: 125 - protein, 7 aa, synthetic construct
YDSYQAS

SEQ ID NO: 126 - protein, 7 aa, synthetic construct
YDSYRAS

SEQ ID NO: 127 - protein, 7 aa, synthetic construct
YDSYRPF

SEQ ID NO: 128 - protein, 7 aa, synthetic construct
YDSYRPG

SEQ ID NO: 129 - protein, 7 aa, synthetic construct
YDSYRSW

SEQ ID NO: 130 - protein, 7 aa, synthetic construct
YDSYTPS

SEQ ID NO: 131 - protein, 7 aa, synthetic construct
YDTFRPT

SEQ ID NO: 132 - protein, 7 aa, synthetic construct
YDVHRPR

SEQ ID NO: 133 - protein, 7 aa, synthetic construct
YDWYRPT

SEQ ID NO: 134 - protein, 7 aa, synthetic construct
YDYFSHS

SEQ ID NO: 135 - protein, 7 aa, synthetic construct
YDYYQSS

SEQ ID NO: 136 - protein, 11 aa, synthetic construct
GAWDYWLGAYV

SEQ ID NO: 137 - protein, 327 aa, synthetic construct
ASTKGPSVFPLAPCSRSTSESTAALGCLVKDYFPEPVTVSWNSGALTSGVHTFPAVLQSSGLYSLSSVVTVPSSSLGTKTYTCNVDHKPSNTKVDKRVESKYGPPCPPCPAPEFLGGPSVFLFPPKPKDTLMISRTPEVTCVVVDVSQEDPEVQFNWYVDGVEVHNAKTKPREEQFNSTYRVVSVLTVLHQDWLNGKEYKCKVSNKGLPSSIEKTISKAKGQPREPQVYTLPPSQEEMTKNQVSLTCLVKGFYPSDIAVEWESNGQPENNYKTTPPVLDSDGSFFLYSRLTVDKSRWQEGNVFSCSVMHEALHNHYTQKSLSLSLGK

SEQ ID NO: 138 - protein, 106 aa, synthetic construct
GQPKAAPSVTLFPPSSEELQANKATLVCLISDFYPGAVTVAWKADSSPVKAGVETTTPSKQSNNKYAASSYLSLTPEQWKSHKSYSCQVTHEGSTVEKTVAPTECS

SEQ ID NO: 139 - protein, 1752 aa, synthetic construct
LEUALALEUSERASPSERARGVALLEUTRPALAPROALAGLUALAHISPROLEUSERPROGLNGLYHISPROALAARGLEUHISARGILEVALPROARGLEUARGASPVALPHEGLYTRPGLYASNLEUTHRCYSPROILECYSLYSGLYLEUPHETHRALAILEASNLEUGLYLEULYSLYSGLUPROASNVALALAARGVALGLYSERVALALAILELYSLEUCYSASNLEULEULYSILEALAPROPROALAVALCYSGLNSERILEVALHISLEUPHEGLUASPASPMETVALGLUVALTRPARGARGSERVALLEUSERPROSERGLUALACYSGLYLEULEULEUGLYSERTHRCYSGLYHISTRPASPILEPHESERSERTRPASNILESERLEUPROTHRVALPROLYSPROPROPROLYSPROPROSERPROPROALAPROGLYALAPROVALSERARGILELEUPHELEUTHRASPLEUHISTRPASPHISASPTYRLEUGLUGLYTHRASPPROASPCYSALAASPPROLEUCYSCYSARGARGGLYSERGLYLEUPROPROALASERARGPROGLYALAGLYTYRTRPGLYGLUTYRSERLYSCYSASPLEUPROLEUARGTHRLEUGLUSERLEULEUSERGLYLEUGLYPROALAGLYPROPHEASPMETVALTYRTRPTHRGLYASPILEPROALAHISASPVALTRPHISGLNTHRARGGLNASPGLNLEUARGALALEUTHRTHRVALTHRALALEUVALARGLYSPHELEUGLYPROVALPROVALTYRPROALAVALGLYASNHISGLUSERTHRPROVALASNSERPHEPROPROPROPHEILEGLUGLYASNHISSERSERARGTRPLEUTYRGLUALAMETALALYSALATRPGLUPROTRPLEUPROALAGLUALALEUARGTHRLEUARGILEGLYGLYPHETYRALALEUSERPROTYRPROGLYLEUARGLEUILESERLEUASNMETASNPHECYSSERARGGLUASNPHETRPLEULEUILEASNSERTHRASPPROALAGLYGLNLEUGLNTRPLEUVALGLYGLULEUGLNALAALAGLUASPARGGLYASPLYSVALHISILEILEGLYHISILEPROPROGLYHISCYSLEULYSSERTRPSERTRPASNTYRTYRARGILEVALALAARGTYRGLUASNTHRLEUALAALAGLNPHEPHEGLYHISTHRHISVALASPGLUPHEGLUVALPHETYRASPGLUGLUTHRLEUSERARGPROLEUALAVALALAPHELEUALAPROSERALATHRTHRTYRILEGLYLEUASNPROGLYTYRARGVALTYRGLNILEASPGLYASNTYRSERGLYSERSERHISVALVALLEUASPHISGLUTHRTYRILELEUASNLEUTHRGLNALAASNILEPROGLYALAILEPROHISTRPGLNLEULEUTYRARGALAARGGLUTHRTYRGLYLEUPROASNTHRLEUPROTHRALATRPHISASNLEUVALTYRARGMETARGGLYASPMETGLNLEUPHEGLNTHRPHETRPPHELEUTYRHISLYSGLYHISPROPROSERGLUPROCYSGLYTHRPROCYSARGLEUALATHRLEUCYSALAGLNLEUSERALAARGALAASPSERPROALALEUCYSARGHISLEUMETPROASPGLYSERLEUPROGLUALAGLNSERLEUTRPPROARGPROLEUPHE

SEQ ID NO: 140 - DNA, 981 bp, synthetic construct
  source 1..981: mol_type = other DNA
gcttctaccaagggacccagcgtgttccctctggctccttgctccagatccacctccgagtctacagctgctctgggctgcctggtcaaggactactttcctgagcctgtgaccgtgtcttggaactctggcgctctgacatccggcgtgcacacctttccagctgtgctgcaatcctccggcctgtactctctgtcctccgtcgtgaccgtgccttctagctctctgggcaccaagacctacacctgtaatgtggaccacaagccttccaacaccaaggtggacaagcgcgtggaatctaagtacggccctccttgtcctccatgtcctgctccagagtttctcggcggaccctccgtgttcctgtttcctccaaagcctaaggacaccctgatgatctctcggacccctgaagtgacctgcgtggtggtggatgtgtcccaagaggatcccgaggtgcagttcaattggtacgtggacggcgtggaagtgcacaacgccaagaccaagcctagagaggaacagttcaactccacctacagagtggtgtccgtgctgaccgtgctgcaccaggattggctgaacggcaaagagtacaagtgcaaggtgtccaacaagggcctgccttccagcatcgaaaagaccatctccaaggccaagggccagcctagggaaccccaggtttacaccctgcctccaagccaagaggaaatgaccaagaaccaggtgtccctgacctgcctcgtgaagggattctacccctccgatatcgccgtggaatgggagtctaatggccagcctgagaacaactacaagacaacccctcctgtgctggactccgacggcagcttcttcctgtattcccgcctgaccgtggacaagtccagatggcaagagggcaacgtgttctcctgctccgtgatgcacgaggccctgcacaatcactacacccagaagtccctgtctctgtccctgggcaag

SEQ ID NO: 141 - DNA, 318 bp, synthetic construct
  source 1..318: mol_type = other DNA
ggccagcccaaagccgccccaagcgtcacactgtttcctccctcatccgaagaactccaggcaaataaggcaactctggtctgtctgatttccgacttctacccaggcgctgtgaccgtcgcatggaaggccgattccagccccgtgaaagcaggagtcgagaccacaactcctagcaagcagtctaacaacaagtacgccgcttctagttatctgagtctgacacccgaacagtggaagagccacaaatcatattcctgccaggtcactcacgaagggtcaactgtggagaaaactgtcgcaccaaccgaatgttcc

SEQ ID NO: 142 - DNA, 291 bp, synthetic construct
  source 1..291: mol_type = other DNA
gccaagacaacacctcctagcgtgtaccctctggctcctggatctgccgctcagaccaatagcatggtcaccctgggctgtctggtcaagggctactttcctgagcctgtgaccgtgacctggaacagcggatctctgtctagcggcgtgcacacctttccagccgtgctgcagagcgatctgtacaccctgagcagcagcgtgaccgtgcctagctctcctagacctagcgagacagtgacctgcaacgtggcccatcctgccagcagcaccaaggtggacaagaaaatc

SEQ ID NO: 143 - DNA, 318 bp, synthetic construct
  source 1..318: mol_type = other DNA
ggccagcctaagagcagccctagcgtgaccctgtttcctccaagcagcgaggaactggaaacaaacaaggccacactcgtgtgcaccatcaccgacttctatcccggcgtggtcaccgtggattggaaggtggacggaacccctgtgacacaaggcatggaaaccacacagcccagcaagcagagcaacaacaagtacatggccagcagctacctgacactgaccgccagagcctgggagagacacagctcctacagctgccaagtgacacacgagggccacaccgtggaaaagtctctgagcagagccgactgcagc